European Patent Application EP 4 424 823 A2, published September 4, 2024. Title: NOVEL ESTERASES AND USES THEREOF. Applicant: CARBIOS. Application EP. The sequence listing filed with the application follows.

SEQUENCE LISTING (7 sequences)

SEQ ID NO: 1 - protein, 258 aa, synthetic construct
  REGION 1..258: note = LC- cutinase
SNPYQRGPNPTRSALTADGPFSVATYTVSRLSVSGFGGGVIYYPTGTSLTFGGIAMSPGYTADASSLAWLGRRLASHGFVVLVINTNSRFDYPDSRASQLSAALNYLRTSSPSAVRARLDANRLAVAGHSMGGGGTLRIAEQNPSLKAAVPLTPWHTDKTFNTSVPVLIVGAEADTVAPVSQHAIPFYQNLPSTTPKVYVELDNASHFAPNSNNAAISVYTISWMKLWVDNDTRYRQFLCNVNDPALSDFRTNNRHCQ

SEQ ID NO: 2 - protein, 258 aa, synthetic construct
  REGION 1..258: note = Poly(ethylene terephthalate) hydrolase
SNPYQRGPNPTRSALTTDGPFSVATYSVSRLSVSGFGGGVIYYPTGTTLTFGGIAMSPGYTADASSLAWLGRRLASHGFVVIVINTNSRLDFPDSRASQLSAALNYLRTSSPSAVRARLDANRLAVAGHSMGGGATLRISEQIPTLKAGVPLTPWHTDKTFNTPVPQLIVGAEADTVAPVSQHAIPFYQNLPSTTPKVYVELDNATHFAPNSPNAAISVYTISWMKLWVDNDTRYRQFLCNVNDPALSDFRSNNRHCQ

SEQ ID NO: 3 - protein, 9 aa, synthetic construct
  REGION 1..9: note = N-terminal peptidique sequence
WASPSVEAQ

SEQ ID NO: 4 - protein, 8 aa, synthetic construct
  REGION 1..8: note = N-terminal peptidique sequence
ASPSVEAQ

SEQ ID NO: 5 - protein, 7 aa, synthetic construct
  REGION 1..7: note = N-terminal peptidique sequence
SPSVEAQ

SEQ ID NO: 6 - protein, 6 aa, synthetic construct
  REGION 1..6: note = N-terminal peptidique sequence
PSVEAQ

SEQ ID NO: 7 - protein, 5 aa, synthetic construct
  REGION 1..5: note = N-terminal peptidique sequence
SVEAQ